European Patent Application EP 4 249 592 A2, published September 27, 2023. Title: Common tumor-specific T cell receptors and antigens. Applicant: HS Diagnomics GMBH. Application EP. The sequence listing filed with the application follows.

SEQUENCE LISTING (158 sequences)

SEQ ID NO: 1 - protein, 13 aa, Homo sapiens
CAASFNQGGKLIF

SEQ ID NO: 2 - protein, 12 aa, Homo sapiens
CAESTPGGKLIF

SEQ ID NO: 3 - protein, 111 aa, Homo sapiens
MEKNPLAAPLLILWFHLDCVSSILNVEQSPQSLHVQEGDSTNFTCSFPSSNFYALHWYRWETAKSPEALFVMTLNGDEKKKGRISATLNTKEGYSYLYIKGSQPEDSATYL

SEQ ID NO: 4 - protein, 151 aa, Homo sapiens
GQGTELSVKPNIQNPDPAVYQLRDSKSSDKSVCLFTDFDSQTNVSQSKDSDVYITDKTVLDMRSMDFKSNSAVAWSNKSDFACANAFNNSIIPEDTFFPSPESSCDVKLVEKSFETDTNLNFQNLSVIGFRILLLKVAGFNLLMTLRLWSS

SEQ ID NO: 5 - protein, 15 aa, Homo sapiens
CVVTAGREYGNKLVF

SEQ ID NO: 6 - protein, 13 aa, Homo sapiens
CAGAYNQGGKLIF

SEQ ID NO: 7 - protein, 15 aa, Homo sapiens
CASSRTSGSLNEQFF

SEQ ID NO: 8 - protein, 13 aa, Homo sapiens
CALLMDSNYQLIW

SEQ ID NO: 9 - protein, 14 aa, Homo sapiens
CASSYDSGTGELFF

SEQ ID NO: 10 - protein, 15 aa, Homo sapiens
CASSIGSGSYNEQFF

SEQ ID NO: 11 - protein, 15 aa, Homo sapiens
CALLSRGSTLGRLYF

SEQ ID NO: 12 - protein, 15 aa, Homo sapiens
CAFMERGSTLGRLYF

SEQ ID NO: 13 - protein, 13 aa, Homo sapiens
CAGSGAGSYQLTF

SEQ ID NO: 14 - protein, 110 aa, Homo sapiens
MKKHLTTFLVILWLYFYRGNGKNQVEQSPQSLIILEGKNCTLQCNYTVSPFSNLRWYKQDTGRGPVSLTIMTFSENTKSNGRYTATLDADTKQSSLHITASQLSDSASYI

SEQ ID NO: 15 - protein, 14 aa, Homo sapiens
CSVGAQGTNEKLFF

SEQ ID NO: 16 - protein, 107 aa, Homo sapiens
MLSLLLLLLGLGSVFSAVISQKPSRDICQRGTSLTIQCQVDSQVTMMFWYRQQPGQSLTLIATANQGSEATYESGFVIDKFPISRPNLTFSTLTVSNMSPEDSSIYL

SEQ ID NO: 17 - protein, 15 aa, Homo sapiens
CASSLTSGSYNEQFF

SEQ ID NO: 18 - protein, 15 aa, Homo sapiens
CAFLTRGSTLGRLYF

SEQ ID NO: 19 - protein, 14 aa, Homo sapiens
CASSEDGMNTEAFF

SEQ ID NO: 20 - protein, 13 aa, Homo sapiens
CASSLGPNYEQYV

SEQ ID NO: 21 - protein, 12 aa, Homo sapiens
CAESSPQGKLIF

SEQ ID NO: 22 - protein, 186 aa, Homo sapiens
GSGTQLSVLEDLNKVFPPEVAVFEPSEAEISHTQKATLVCLATGFFPDHVELSWWVNGKEVHSGVSTDPQPLKEQPALNDSRYCLSSRLRVSATFWQNPRNHFRCQVQFYGLSENDEWTQDRAKPVTQIVSAEAWGRADCGFTSVSYQQGVLSATILYEILLGKATLYAVLVSALVLMAMVKRKDF

SEQ ID NO: 23 - protein, 110 aa, Homo sapiens
MGTSLLCWVVLGFLGTDHTGAGVSQSPRYKVTKRGQDVALRCDPISGHVSLYWYRQALGQGPEFLTYFNYEAQQDKSGLPNDRFSAERPEGSISTLTIQRTEQRDSAMYR

SEQ ID NO: 24 - protein, 12 aa, Homo sapiens
CAESTSRGKLIF

SEQ ID NO: 25 - protein, 15 aa, Homo sapiens
CVVSAGREYGNKLVF

SEQ ID NO: 26 - protein, 15 aa, Homo sapiens
CAPLPRGSTLGRLYF

SEQ ID NO: 27 - protein, 14 aa, Homo sapiens
CSVGSGGTNEKLFF

SEQ ID NO: 28 - protein, 14 aa, Homo sapiens
CASSLDGMNTEAFF

SEQ ID NO: 29 - protein, 12 aa, Homo sapiens
CALSDTGNQFYF

SEQ ID NO: 30 - protein, 109 aa, Homo sapiens
MGTRLFFYVALCLLWAGHRDAGITQSPRYKITETGRQVTLMCHQTWSHSYMFWYRQDLGHGLRLIYYSAAADITDKGEVPDGYVVSRSKTENFPLTLESATRSQTSVYF

SEQ ID NO: 31 - protein, 14 aa, Homo sapiens
CSVGTGGTNEKLFF

SEQ ID NO: 32 - protein, 12 aa, Homo sapiens
CAESTPRGRLMF

SEQ ID NO: 33 - protein, 188 aa, Homo sapiens
GPGTRLTVTEDLKNVFPPEVAVFEPSEAEISHTQKATLVCLATGFYPDHVELSWWVNGKEVHSGVSTDPQPLKEQPALNDSRYCLSSRLRVSATFWQNPRNHFRCQVQFYGLSENDEWTQDRAKPVTQIVSAEAWGRADCGFTSESYQQGVLSATILYEILLGKATLYAVLVSALVLMAMVKRKDSRG

SEQ ID NO: 34 - protein, 188 aa, Homo sapiens
GEGSRLTVLEDLKNVFPPKVAVFEPSEAEISHTQKATLVCLATGFYPDHVELSWWVNGKEVHSGVSTDPQPLKEQPALNDSRYCLSSRLRVSATFWQNPRNHFRCQVQFYGLSENDEWTQDRAKPVTQIVSAEAWGRADCGFTSESYQQGVLSATILYEILLGKATLYAVLVSALVLMAMVKRKDSRG

SEQ ID NO: 35 - protein, 106 aa, Homo sapiens
MLLITSMLVLWMQLSQVNGQQVMQIPQYQHVQEGEDFTTYCNSSTTLSNIQWYKQRPGGHPVFLIQLVKSGEVKKQKRLTFQFGEAKKNSSLHITATQTTDVGTYF

SEQ ID NO: 36 - protein, 109 aa, Homo sapiens
MSNQVLCCVVLCFLGANTVDGGITQSPKYLFRKEGQNVTLSCEQNLNHDAMYWYRQDPGQGLRLIYYSQIVNDFQKGDIAEGYSVSREKKESFPLTVTSAQKNPTAFYL

SEQ ID NO: 37 - protein, 186 aa, Homo sapiens
GQGTRLTVVEDLNKVFPPEVAVFEPSEAEISHTQKATLVCLATGFFPDHVELSWWVNGKEVHSGVSTDPQPLKEQPALNDSRYCLSSRLRVSATFWQNPRNHFRCQVQFYGLSENDEWTQDRAKPVTQIVSAEAWGRADCGFTSVSYQQGVLSATILYEILLGKATLYAVLVSALVLMAMVKRKDF

SEQ ID NO: 38 - protein, 13 aa, Homo sapiens
CASSPGPNYEQYF

SEQ ID NO: 39 - protein, 109 aa, Homo sapiens
MSIGLLCCAALSLLWAGPVNAGVTQTPKFQVLKTGQSMTLQCAQDMNHEYMSWYRQDPGMGLRLIHYSVGAGITDQGEVPNGYNVSRSTTEDFPLRLLSAAPSQTSVYF

SEQ ID NO: 40 - protein, 151 aa, Homo sapiens
GKGTKLSVIPNIQNPDPAVYQLRDSKSSDKSVCLFTDFDSQTNVSQSKDSDVYITDKTVLDMRSMDFKSNSAVAWSNKSDFACANAFNNSIIPEDTFFPSPESSCDVKLVEKSFETDTNLNFQNLSVIGFRILLLKVAGFNLLMTLRLWSS

SEQ ID NO: 41 - protein, 13 aa, Homo sapiens
CASSAGPNYEQYF

SEQ ID NO: 42 - protein, 15 aa, Homo sapiens
CASSLTSGNYNEQFF

SEQ ID NO: 43 - protein, 109 aa, Homo sapiens
MGSRLLCWVLLCLLGAGPVKAGVTQTPRYLIKTRGQQVTLSCSPISGHRSVSWYQQTPGQGLQFLFEYFSETQRNKGNFPGRFSGRQFSNSRSEMNVSTLELGDSALYL

SEQ ID NO: 44 - protein, 15 aa, Homo sapiens
CASTVTSGSYNEQFF

SEQ ID NO: 45 - protein, 14 aa, Homo sapiens
CASSPDGMNTEAFF

SEQ ID NO: 46 - protein, 15 aa, Homo sapiens
CVVSVGREYGNKLVF

SEQ ID NO: 47 - protein, 14 aa, Homo sapiens
CASSFVSGTDTQYF

SEQ ID NO: 48 - protein, 151 aa, Homo sapiens
GTGTRLQVTLDIQNPDPAVYQLRDSKSSDKSVCLFTDFDSQTNVSQSKDSDVYITDKTVLDMRSMDFKSNSAVAWSNKSDFACANAFNNSIIPEDTFFPSPESSCDVKLVEKSFETDTNLNFQNLSVIGFRILLLKVAGFNLLMTLRLWSS

SEQ ID NO: 49 - protein, 111 aa, Homo sapiens
MLTASLLRAVIASICVVSSMAQKVTQAQTEISVVEKEDVTLDCVYETRDTTYYLFWYKQPPSGELVFLIRRNSFDEQNEISGRYSWNFQKSTSSFNFTITASQVVDSAVYF

SEQ ID NO: 50 - protein, 151 aa, Homo sapiens
GAGTILRVKSYIQNPDPAVYQLRDSKSSDKSVCLFTDFDSQTNVSQSKDSDVYITDKTVLDMRSMDFKSNSAVAWSNKSDFACANAFNNSIIPEDTFFPSPESSCDVKLVEKSFETDTNLNFQNLSVIGFRILLLKVAGFNLLMTLRLWSS

SEQ ID NO: 51 - protein, 13 aa, Homo sapiens
CAVLMDSNYQLIW

SEQ ID NO: 52 - protein, 12 aa, Homo sapiens
CALSETGNQFYF

SEQ ID NO: 53 - protein, 151 aa, Homo sapiens
GRGTQLTVWPDIQNPDPAVYQLRDSKSSDKSVCLFTDFDSQTNVSQSKDSDVYITDKTVLDMRSMDFKSNSAVAWSNKSDFACANAFNNSIIPEDTFFPSPESSCDVKLVEKSFETDTNLNFQNLSVIGFRILLLKVAGFNLLMTLRLWSS

SEQ ID NO: 54 - protein, 115 aa, Homo sapiens
MAMLLGASVLILWLQPDWVNSQQKNDDQQVKQNSPSLSVQEGRISILNCDYTNSMFDYFLWYKKYPAEGPTFLISISSIKDKNEDGRFTVFLNKSAKHLSLHIVPSQPGDSAVYF

SEQ ID NO: 55 - protein, 15 aa, Homo sapiens
CAFMPRGSTLGRLYF

SEQ ID NO: 56 - protein, 188 aa, Homo sapiens
GPGTRLTVLEDLKNVFPPKVAVFEPSEAEISHTQKATLVCLATGFYPDHVELSWWVNGKEVHSGVSTDPQPLKEQPALNDSRYCLSSRLRVSATFWQNPRNHFRCQVQFYGLSENDEWTQDRAKPVTQIVSAEAWGRADCGFTSESYQQGVLSATILYEILLGKATLYAVLVSALVLMAMVKRKDSRG

SEQ ID NO: 57 - protein, 109 aa, Homo sapiens
MKTFAGFSFLFLWLQLDCMSRGEDVEQSLFLSVREGDSSVINCTYTDSSSTYLYWYKQEPGAGLQLLTYIFSNMDMKQDQRLTVLLNKKDKHLSLRIADTQTGDSAIYF

SEQ ID NO: 58 - protein, 15 aa, Homo sapiens
CAFMARGSTLGRLYF

SEQ ID NO: 59 - protein, 13 aa, Homo sapiens
CAASSNQGGKLIF

SEQ ID NO: 60 - protein, 14 aa, Homo sapiens
CASSSDGMNTEAFF

SEQ ID NO: 61 - protein, 16 aa, Homo sapiens
CASSLEGQASSYEQYF

SEQ ID NO: 62 - protein, 14 aa, Homo sapiens
CAARNTGTASKLTF

SEQ ID NO: 63 - protein, 14 aa, Homo sapiens
CAARLTGTASKLTF

SEQ ID NO: 64 - protein, 109 aa, Homo sapiens
MGIRLLCRVAFCFLAVGLVDVKVTQSSRYLVKRTGEKVFLECVQDMDHENMFWYRQDPGLGLRLIYFSYDVKMKEKGDIPEGYSVSREKKERFSLILESASTNQTSMYL

SEQ ID NO: 65 - protein, 13 aa, Homo sapiens
CAGAGAGSYQLTF

SEQ ID NO: 66 - protein, 151 aa, Homo sapiens
GTGTSLTVIPNIQNPDPAVYQLRDSKSSDKSVCLFTDFDSQTNVSQSKDSDVYITDKTVLDMRSMDFKSNSAVAWSNKSDFACANAFNNSIIPEDTFFPSPESSCDVKLVEKSFETDTNLNFQNLSVIGFRILLLKVAGFNLLMTLRLWSS

SEQ ID NO: 67 - protein, 108 aa, Homo sapiens [sequence omitted]

SEQ ID NO: 68 - protein, 108 aa, Homo sapiens
METLLGLLILWLQLQWVSSKQEVTQIPAALSVPEGENLVLNCSFTDSAIYNLQWFRQDPGKGLTSLLLIQSSQREQTSGRLNASLDKSSGRSTLYIAASQPGDSATYL

SEQ ID NO: 69 - protein, 188 aa, Homo sapiens
GPGTRLTVTEDLKNVFPPKVAVFEPSEAEISHTQKATLVCLATGFYPDHVELSWWVNGKEVHSGVSTDPQPLKEQPALNDSRYCLSSRLRVSATFWQNPRNHFRCQVQFYGLSENDEWTQDRAKPVTQIVSAEAWGRADCGFTSESYQQGVLSATILYEILLGKATLYAVLVSALVLMAMVKRKDSRG

SEQ ID NO: 70 - protein, 151 aa, Homo sapiens
GAGTKLIIKPDIQNPDPAVYQLRDSKSSDKSVCLFTDFDSQTNVSQSKDSDVYITDKTVLDMRSMDFKSNSAVAWSNKSDFACANAFNNSIIPEDTFFPSPESSCDVKLVEKSFETDTNLNFQNLSVIGFRILLLKVAGFNLLMTLRLWSS

SEQ ID NO: 71 - protein, 14 aa, Homo sapiens
CAARNAGTASKLTF

SEQ ID NO: 72 - protein, 14 aa, Homo sapiens
CASSFLAGTDTQYF

SEQ ID NO: 73 - protein, 14 aa, Homo sapiens
CASSFLSGTDTQYF

SEQ ID NO: 74 - DNA, 39 bp, Homo sapiens
  source 1..39: mol_type = other DNA
tgtgccagcagccccggacccaactacgagcagtacttc

SEQ ID NO: 75 - DNA, 48 bp, Homo sapiens
  source 1..48: mol_type = other DNA
tgcgccagcagcttggaaggacaggcgagctcctacgagcagtacttc

SEQ ID NO: 76 - DNA, 456 bp, Homo sapiens
  source 1..456: mol_type = other DNA
gggacagggacaagtttgacggtcattccaaatatccagaaccctgaccctgccgtgtaccagctgagagactctaaatccagtgacaagtctgtctgcctattcaccgattttgattctcaaacaaatgtgtcacaaagtaaggattctgatgtgtatatcacagacaaaactgtgctagacatgaggtctatggacttcaagagcaacagtgctgtggcctggagcaacaaatctgactttgcatgtgcaaacgccttcaacaacagcattattccagaagacaccttcttccccagcccagaaagttcctgtgatgtcaagctggtcgagaaaagctttgaaacagatacgaacctaaactttcaaaacctgtcagtgattgggttccgaatcctcctcctgaaagtggccgggtttaatctgctcatgacgctgcggctgtggtccagctga

SEQ ID NO: 77 - DNA, 42 bp, Homo sapiens
  source 1..42: mol_type = other DNA
tgcgccagcagtgaggacggcatgaacactgaagctttcttt

SEQ ID NO: 78 - DNA, 327 bp, Homo sapiens
  source 1..327: mol_type = other DNA
atgggcaccaggctcttcttctatgtggccctttgtctgctgtgggcaggacacagggatgctggaatcacccagagcccaagatacaagatcacagagacaggaaggcaggtgaccttgatgtgtcaccagacttggagccacagctatatgttctggtatcgacaagacctgggacatgggctgaggctgatctattactcagcagctgctgatattacagataaaggagaagtccccgatggctatgttgtctccagatccaagacagagaatttccccctcactctggagtcagctacccgctcccagacatctgtgtatttc

SEQ ID NO: 79 - DNA, 345 bp, Homo sapiens
  source 1..345: mol_type = other DNA
atggccatgctcctgggggcatcagtgctgattctgtggcttcagccagactgggtaaacagtcaacagaagaatgatgaccagcaagttaagcaaaattcaccatccctgagcgtccaggaaggaagaatttctattctgaactgtgactatactaacagcatgtttgattatttcctatggtacaaaaaataccctgctgaaggtcctacattcctgatatctataagttccattaaggataaaaatgaagatggaagattcactgtcttcttaaacaaaagtgccaagcacctctctctgcacattgtgccctcccagcctggagactctgcagtgtacttc

SEQ ID NO: 80 - DNA, 567 bp, Homo sapiens
  source 1..567: mol_type = other DNA
gggccgggcaccaggctcacggtcacagaggacctgaaaaacgtgttcccacccaaggtcgctgtgtttgagccatcagaagcagagatctcccacacccaaaaggccacactggtgtgcctggccacaggcttctaccccgaccacgtggagctgagctggtgggtgaatgggaaggaggtgcacagtggggtcagcacagacccgcagcccctcaaggagcagcccgccctcaatgactccagatactgcctgagcagccgcctgagggtctcggccaccttctggcagaacccccgcaaccacttccgctgtcaagtccagttctacgggctctcggagaatgacgagtggacccaggatagggccaaacctgtcacccagatcgtcagcgccgaggcctggggtagagcagactgtggcttcacctccgagtcttaccagcaaggggtcctgtctgccaccatcctctatgagatcttgctagggaaggccaccttgtatgccgtgctggtcagtgccctcgtgctgatggccatggtcaagagaaaggattccagaggctag

SEQ ID NO: 81 - DNA, 561 bp, Homo sapiens
  source 1..561: mol_type = other DNA
ggcagtggaacccagctctctgtcttggaggacctgaacaaggtgttcccacccgaggtcgctgtgtttgagccatcagaagcagagatctcccacacccaaaaggccacactggtgtgcctggccacaggcttcttccctgaccacgtggagctgagctggtgggtgaatgggaaggaggtgcacagtggggtcagcacggacccgcagcccctcaaggagcagcccgccctcaatgactccagatactgcctgagcagccgcctgagggtctcggccaccttctggcagaacccccgcaaccacttccgctgtcaagtccagttctacgggctctcggagaatgacgagtggacccaggatagggccaaacccgtcacccagatcgtcagcgccgaggcctggggtagagcagactgtggctttacctcggtgtcctaccagcaaggggtcctgtctgccaccatcctctatgagatcctgctagggaaggccaccctgtatgctgtgctggtcagcgcccttgtgttgatggccatggtcaagagaaaggatttctga

SEQ ID NO: 82 - DNA, 45 bp, Homo sapiens
  source 1..45: mol_type = other DNA
tgtgtggtgagcgttggaagggaatatggaaacaaactggtcttt

SEQ ID NO: 83 - DNA, 42 bp, Homo sapiens
  source 1..42: mol_type = other DNA
tgcgccagcagcttggacggaatgaacactgaagctttcttt

SEQ ID NO: 84 - DNA, 42 bp, Homo sapiens
  source 1..42: mol_type = other DNA
tgcagcgttggggctcagggaactaatgaaaaactgtttttt

SEQ ID NO: 85 - DNA, 39 bp, Homo sapiens
  source 1..39: mol_type = other DNA
tgtgcaggggcgtataaccagggaggaaagcttatcttc

SEQ ID NO: 86 - DNA, 567 bp, Homo sapiens
  source 1..567: mol_type = other DNA
ggcccaggcacccggctgacagtgctcgaggacctgaaaaacgtgttcccacccaaggtcgctgtgtttgagccatcagaagcagagatctcccacacccaaaaggccacactggtgtgcctggccacaggcttctaccccgaccacgtggagctgagctggtgggtgaatgggaaggaggtgcacagtggggtcagcacagacccgcagcccctcaaggagcagcccgccctcaatgactccagatactgcctgagcagccgcctgagggtctcggccaccttctggcagaacccccgcaaccacttccgctgtcaagtccagttctacgggctctcggagaatgacgagtggacccaggatagggccaaacctgtcacccagatcgtcagcgccgaggcctggggtagagcagactgtggcttcacctccgagtcttaccagcaaggggtcctgtctgccaccatcctctatgagatcttgctagggaaggccaccttgtatgccgtgctggtcagtgccctcgtgctgatggccatggtcaagagaaaggattccagaggctag

SEQ ID NO: 87 - DNA, 456 bp, Homo sapiens
  source 1..456: mol_type = other DNA
ggacagggaacggagttatctgtgaaacccaatatccagaaccctgaccctgccgtgtaccagctgagagactctaaatccagtgacaagtctgtctgcctattcaccgattttgattctcaaacaaatgtgtcacaaagtaaggattctgatgtgtatatcacagacaaaactgtgctagacatgaggtctatggacttcaagagcaacagtgctgtggcctggagcaacaaatctgactttgcatgtgcaaacgccttcaacaacagcattattccagaagacaccttcttccccagcccagaaagttcctgtgatgtcaagctggtcgagaaaagctttgaaacagatacgaacctaaactttcaaaacctgtcagtgattgggttccgaatcctcctcctgaaagtggccgggtttaatctgctcatgacgctgcggctgtggtccagctga

SEQ ID NO: 88 - DNA, 42 bp, Homo sapiens
  source 1..42: mol_type = other DNA
tgtgccagcagttttgtgagcggcacagatacgcagtatttt

SEQ ID NO: 89 - DNA, 42 bp, Homo sapiens
  source 1..42: mol_type = other DNA
tgcagcgtcggaacaggggggactaatgaaaaactgtttttt

SEQ ID NO: 90 - DNA, 39 bp, Homo sapiens
  source 1..39: mol_type = other DNA
tgtgctttactcatggatagcaactatcagttaatctgg

SEQ ID NO: 91 - DNA, 36 bp, Homo sapiens
  source 1..36: mol_type = other DNA
tgtgctctgagtgagaccggtaaccagttctatttt

SEQ ID NO: 92 - DNA, 42 bp, Homo sapiens
  source 1..42: mol_type = other DNA
tgcgccagcagcccggacggaatgaacactgaagctttcttt

SEQ ID NO: 93 - DNA, 45 bp, Homo sapiens
  source 1..45: mol_type = other DNA
tgtgccagtagtcggactagcgggagtcttaatgagcagttcttc

SEQ ID NO: 94 - DNA, 45 bp, Homo sapiens
  source 1..45: mol_type = other DNA
tgtgtggtgagcgccgggagggaatatggaaacaaactggtcttt

SEQ ID NO: 95 - DNA, 45 bp, Homo sapiens
  source 1..45: mol_type = other DNA
tgtgccagtagtctcactagcggttcctacaatgagcagttcttc

SEQ ID NO: 96 - DNA, 330 bp, Homo sapiens
  source 1..330: mol_type = other DNA
atgggcaccagtctcctatgctgggtggtcctgggtttcctagggacagatcacacaggtgctggagtctcccagtctcccaggtacaaagtcacaaagaggggacaggatgtagctctcaggtgtgatccaatttcgggtcatgtatccctttattggtaccgacaggccctggggcagggcccagagtttctgacttacttcaattatgaagcccaacaagacaaatcagggctgcccaatgatcggttctctgcagagaggcctgagggatccatctccactctgacgatccagcgcacagagcagcgggactcggccatgtatcgc

SEQ ID NO: 97 - DNA, 327 bp, Homo sapiens
  source 1..327: mol_type = other DNA
atgggaatcaggctcctctgtcgtgtggccttttgtttcctggctgtaggcctcgtagatgtgaaagtaacccagagctcgagatatctagtcaaaaggacgggagagaaagtttttctggaatgtgtccaggatatggaccatgaaaatatgttctggtatcgacaagacccaggtctggggctacggctgatctatttctcatatgatgttaaaatgaaagaaaaaggagatattcctgaggggtacagtgtctctagagagaagaaggagcgcttctccctgattctggagtccgccagcaccaaccagacatctatgtacctc

SEQ ID NO: 98 - DNA, 42 bp, Homo sapiens
  source 1..42: mol_type = other DNA
tgcgccagcagtttggacgggatgaacactgaagctttcttt

SEQ ID NO: 99 - DNA, 36 bp, Homo sapiens
  source 1..36: mol_type = other DNA
tgtgctctgagtgacaccggtaaccagttctatttt

SEQ ID NO: 100 - DNA, 36 bp, Homo sapiens
  source 1..36: mol_type = other DNA
tgtgcagagagtacctccaggggaaagcttatcttc

SEQ ID NO: 101 - DNA, 42 bp, Homo sapiens
  source 1..42: mol_type = other DNA
tgtgccagcagttttctttcaggcacagatacgcagtatttt

SEQ ID NO: 102 - DNA, 45 bp, Homo sapiens
  source 1..45: mol_type = other DNA
tgtgcccccctcccgagaggctcaaccctggggaggctatacttt

SEQ ID NO: 103 - DNA, 561 bp, Homo sapiens
  source 1..561: mol_type = other DNA
ggacaaggcaccagactcacagttgtagaggacctgaacaaggtgttcccacccgaggtcgctgtgtttgagccatcagaagcagagatctcccacacccaaaaggccacactggtgtgcctggccacaggcttcttccctgaccacgtggagctgagctggtgggtgaatgggaaggaggtgcacagtggggtcagcacggacccgcagcccctcaaggagcagcccgccctcaatgactccagatactgcctgagcagccgcctgagggtctcggccaccttctggcagaacccccgcaaccacttccgctgtcaagtccagttctacgggctctcggagaatgacgagtggacccaggatagggccaaacccgtcacccagatcgtcagcgccgaggcctggggtagagcagactgtggctttacctcggtgtcctaccagcaaggggtcctgtctgccaccatcctctatgagatcctgctagggaaggccaccctgtatgctgtgctggtcagcgcccttgtgttgatggccatggtcaagagaaaggatttctga

SEQ ID NO: 104 - DNA, 327 bp, Homo sapiens
  source 1..327: mol_type = other DNA
atgaagacatttgctggattttcgttcctgtttttgtggctgcagctggactgtatgagtagaggagaggatgtggagcagagtcttttcctgagtgtccgagagggagacagctccgttataaactgcacttacacagacagctcctccacctacttatactggtataagcaagaacctggagcaggtctccagttgctgacgtatattttttcaaatatggacatgaaacaagaccaaagactcactgttctattgaataaaaaggataaacatctgtctctgcgcattgcagacacccagactggggactcagctatctacttc

SEQ ID NO: 105 - DNA, 318 bp, Homo sapiens
  source 1..318: mol_type = other DNA
atgctactcatcacatcaatgttggtcttatggatgcaattgtcacaggtgaatggacaacaggtaatgcaaattcctcagtaccagcatgtacaagaaggagaagacttcaccacgtactgcaattcctcaactactttaagcaatatacagtggtataagcaaaggcctggtggacatcccgtttttttgatacagttagtgaagagtggagaagtgaagaagcagaaaagactgacatttcagtttggagaagcaaaaaagaacagctccctgcacatcacagccacccagactacagatgtaggaacctacttc

SEQ ID NO: 106 - DNA, 39 bp, Homo sapiens
  source 1..39: mol_type = other DNA
tgtgcagcaagttttaaccagggaggaaagcttatcttc

SEQ ID NO: 107 - DNA, 42 bp, Homo sapiens
  source 1..42: mol_type = other DNA
tgcgccagcagttccgacgggatgaacactgaagctttcttt

SEQ ID NO: 108 - DNA, 324 bp, Homo sapiens
  source 1..324: mol_type = other DNA
atgacatccattcgagctgtatttatattcctgtggctgcagctggacttggtgaatggagagaatgtggagcagcatccttcaaccctgagtgtccaggagggagacagcgctgttatcaagtgtacttattcagacagtgcctcaaactacttcccttggtataagcaagaacttggaaaaagacctcagcttattatagacattcgttcaaatgtgggcgaaaagaaagaccaacgaattgctgttacattgaacaagacagccaaacatttctccctgcacatcacagagacccaacctgaagactcggctgtctacttc

SEQ ID NO: 109 - DNA, 327 bp, Homo sapiens
  source 1..327: mol_type = other DNA
atgagcaaccaggtgctctgctgtgtggtcctttgtttcctgggagcaaacaccgtggatggtggaatcactcagtccccaaagtacctgttcagaaaggaaggacagaatgtgaccctgagttgtgaacagaatttgaaccacgatgccatgtactggtaccgacaggacccagggcaagggctgagattgatctactactcacagatagtaaatgactttcagaaaggagatatagctgaagggtacagcgtctctcgggagaagaaggaatcctttcctctcactgtgacatcggcccaaaagaacccgacagctttctatctc

SEQ ID NO: 110 - DNA, 36 bp, Homo sapiens
  source 1..36: mol_type = other DNA
tgtgcagagtcaactccccggggcagactcatgttt

SEQ ID NO: 111 - DNA, 456 bp, Homo sapiens
  source 1..456: mol_type = other DNA
ggcgctgggaccaagctaattataaagccagatatccagaaccctgaccctgccgtgtaccagctgagagactctaaatccagtgacaagtctgtctgcctattcaccgattttgattctcaaacaaatgtgtcacaaagtaaggattctgatgtgtatatcacagacaaaactgtgctagacatgaggtctatggacttcaagagcaacagtgctgtggcctggagcaacaaatctgactttgcatgtgcaaacgccttcaacaacagcattattccagaagacaccttcttccccagcccagaaagttcctgtgatgtcaagctggtcgagaaaagctttgaaacagatacgaacctaaactttcaaaacctgtcagtgattgggttccgaatcctcctcctgaaagtggccgggtttaatctgctcatgacgctgcggctgtggtccagctga

SEQ ID NO: 112 - DNA, 321 bp, Homo sapiens
  source 1..321: mol_type = other DNA
atgctgagtcttctgctccttctcctgggactaggctctgtgttcagtgctgtcatctctcaaaagccaagcagggatatctgtcaacgtggaacctccctgacgatccagtgtcaagtcgatagccaagtcaccatgatgttctggtaccgtcagcaacctggacagagcctgacactgatcgcaactgcaaatcagggctctgaggccacatatgagagtggatttgtcattgacaagtttcccatcagccgcccaaacctaacattctcaactctgactgtgagcaacatgagccctgaagacagcagcatatatctc

SEQ ID NO: 113 - DNA, 567 bp, Homo sapiens
  source 1..567: mol_type = other DNA
gggccagggacacggctcaccgtgctagaggacctgaaaaacgtgttcccacccaaggtcgctgtgtttgagccatcagaagcagagatctcccacacccaaaaggccacactggtgtgcctggccacaggcttctaccccgaccacgtggagctgagctggtgggtgaatgggaaggaggtgcacagtggggtcagcacagacccgcagcccctcaaggagcagcccgccctcaatgactccagatactgcctgagcagccgcctgagggtctcggccaccttctggcagaacccccgcaaccacttccgctgtcaagtccagttctacgggctctcggagaatgacgagtggacccaggatagggccaaacctgtcacccagatcgtcagcgccgaggcctggggtagagcagactgtggcttcacctccgagtcttaccagcaaggggtcctgtctgccaccatcctctatgagatcttgctagggaaggccaccttgtatgccgtgctggtcagtgccctcgtgctgatggccatggtcaagagaaaggattccagaggctag

SEQ ID NO: 114 - DNA, 36 bp, Homo sapiens
  source 1..36: mol_type = other DNA
tgtgctctgagtgaaaccggtaaccagttctatttt

SEQ ID NO: 115 - DNA, 42 bp, Homo sapiens
  source 1..42: mol_type = other DNA
tgtgccagcagtttcgtcagcggcacagatacgcagtatttt

SEQ ID NO: 116 - DNA, 327 bp, Homo sapiens
  source 1..327: mol_type = other DNA
atgggctccaggctgctctgttgggtgctgctttgtctcctgggagcaggcccagtaaaggctggagtcactcaaactccaagatatctgatcaaaacgagaggacagcaagtgacactgagctgctcccctatctctgggcataggagtgtatcctggtaccaacagaccccaggacagggccttcagttcctctttgaatacttcagtgagacacagagaaacaaaggaaacttccctggtcgattctcagggcgccagttctctaactctcgctctgagatgaatgtgagcaccttggagctgggggactcggccctttatctt

SEQ ID NO: 117 - DNA, 45 bp, Homo sapiens
  source 1..45: mol_type = other DNA
tgtgccagtaccgtaacaagcgggagctacaatgagcagttcttc

SEQ ID NO: 118 - DNA, 45 bp, Homo sapiens
  source 1..45: mol_type = other DNA
tgtgccagtagtattggcagcgggagttacaatgagcagttcttc

SEQ ID NO: 119 - DNA, 45 bp, Homo sapiens
  source 1..45: mol_type = other DNA
tgtgcctttcttaccagaggctcaaccctggggaggctatacttt

SEQ ID NO: 120 - DNA, 39 bp, Homo sapiens
  source 1..39: mol_type = other DNA
tgtgctgtcctaatggatagcaactatcagttaatctgg

SEQ ID NO: 121 - DNA, 42 bp, Homo sapiens
  source 1..42: mol_type = other DNA
tgtgccagcagttatgacagcggaaccggggagctgtttttt

SEQ ID NO: 122 - DNA, 45 bp, Homo sapiens
  source 1..45: mol_type = other DNA
tgtgtggtgagcgcggggagggaatatggaaacaaactggtcttt

SEQ ID NO: 123 - DNA, 39 bp, Homo sapiens
  source 1..39: mol_type = other DNA
tgtgcagcaagtagtaaccagggaggaaagcttatcttc

SEQ ID NO: 124 - DNA, 45 bp, Homo sapiens
  source 1..45: mol_type = other DNA
tgtgcctttatggagagaggctcaaccctggggaggctatacttt

SEQ ID NO: 125 - DNA, 39 bp, Homo sapiens
  source 1..39: mol_type = other DNA
tgtgccagcagcttaggcccgaattacgagcagtacgtc

SEQ ID NO: 126 - DNA, 39 bp, Homo sapiens
  source 1..39: mol_type = other DNA
tgtgcaggatctggggctgggagttaccaactcactttc

SEQ ID NO: 127 - DNA, 42 bp, Homo sapiens
  source 1..42: mol_type = other DNA
tgcagcgttgggacagggggaactaatgaaaaactgtttttt

SEQ ID NO: 128 - DNA, 567 bp, Homo sapiens
  source 1..567: mol_type = other DNA
ggagaaggctctaggctgaccgtactggaggacctgaaaaacgtgttcccacccaaggtcgctgtgtttgagccatcagaagcagagatctcccacacccaaaaggccacactggtgtgcctggccacaggcttctaccccgaccacgtggagctgagctggtgggtgaatgggaaggaggtgcacagtggggtcagcacagacccgcagcccctcaaggagcagcccgccctcaatgactccagatactgcctgagcagccgcctgagggtctcggccaccttctggcagaacccccgcaaccacttccgctgtcaagtccagttctacgggctctcggagaatgacgagtggacccaggatagggccaaacctgtcacccagatcgtcagcgccgaggcctggggtagagcagactgtggcttcacctccgagtcttaccagcaaggggtcctgtctgccaccatcctctatgagatcttgctagggaaggccaccttgtatgccgtgctggtcagtgccctcgtgctgatggccatggtcaagagaaaggattccagaggctag

SEQ ID NO: 129 - DNA, 42 bp, Homo sapiens
  source 1..42: mol_type = other DNA
tgcgccagcagcttggacggcatgaacactgaagctttcttt

SEQ ID NO: 130 - DNA, 45 bp, Homo sapiens
  source 1..45: mol_type = other DNA
tgtgtggtgaccgcggggagggaatatggaaacaaactggtcttt

SEQ ID NO: 131 - DNA, 333 bp, Homo sapiens
  source 1..333: mol_type = other DNA
atggagaagaatcctttggcagccccattactaatcctctggtttcatcttgactgcgtgagcagcatactgaacgtggaacaaagtcctcagtcactgcatgttcaggagggagacagcaccaatttcacctgcagcttcccttccagcaatttttatgccttacactggtacagatgggaaactgcaaaaagccccgaggccttgtttgtaatgactttaaatggggatgaaaagaagaaaggacgaataagtgccactcttaataccaaggagggttacagctatttgtacatcaaaggatcccagcctgaagactcagccacatacctc

SEQ ID NO: 132 - DNA, 45 bp, Homo sapiens
  source 1..45: mol_type = other DNA
tgtgccttattaagcagaggctcaaccctggggaggctatacttt

SEQ ID NO: 133 - DNA, 42 bp, Homo sapiens
  source 1..42: mol_type = other DNA
tgtgccagcagtttcgtttcaggcacagatacgcagtatttt

SEQ ID NO: 134 - DNA, 45 bp, Homo sapiens
  source 1..45: mol_type = other DNA
tgtgcctttatggccagaggctcaaccctggggaggctatacttt

SEQ ID NO: 135 - DNA, 39 bp, Homo sapiens
  source 1..39: mol_type = other DNA
tgtgctggggctggggctgggagttaccaactcactttc

SEQ ID NO: 136 - DNA, 42 bp, Homo sapiens
  source 1..42: mol_type = other DNA
tgtgccagcagtttcctagcgggcacagatacgcagtatttt

SEQ ID NO: 137 - DNA, 456 bp, Homo sapiens
  source 1..456: mol_type = other DNA
ggcgcaggaaccattctgagagtcaagtcctatatccagaaccctgaccctgccgtgtaccagctgagagactctaaatccagtgacaagtctgtctgcctattcaccgattttgattctcaaacaaatgtgtcacaaagtaaggattctgatgtgtatatcacagacaaaactgtgctagacatgaggtctatggacttcaagagcaacagtgctgtggcctggagcaacaaatctgactttgcatgtgcaaacgccttcaacaacagcattattccagaagacaccttcttccccagcccagaaagttcctgtgatgtcaagctggtcgagaaaagctttgaaacagatacgaacctaaactttcaaaacctgtcagtgattgggttccgaatcctcctcctgaaagtggccgggtttaatctgctcatgacgctgcggctgtggtccagctga

SEQ ID NO: 138 - DNA, 456 bp, Homo sapiens
  source 1..456: mol_type = other DNA
ggaagaggaactcagttgactgtctggcctgatatccagaaccctgaccctgccgtgtaccagctgagagactctaaatccagtgacaagtctgtctgcctattcaccgattttgattctcaaacaaatgtgtcacaaagtaaggattctgatgtgtatatcacagacaaaactgtgctagacatgaggtctatggacttcaagagcaacagtgctgtggcctggagcaacaaatctgactttgcatgtgcaaacgccttcaacaacagcattattccagaagacaccttcttccccagcccagaaagttcctgtgatgtcaagctggtcgagaaaagctttgaaacagatacgaacctaaactttcaaaacctgtcagtgattgggttccgaatcctcctcctgaaagtggccgggtttaatctgctcatgacgctgcggctgtggtccagctga

SEQ ID NO: 139 - DNA, 39 bp, Homo sapiens
  source 1..39: mol_type = other DNA
tgtgccagcagtgcagggcccaattacgagcagtacttc

SEQ ID NO: 140 - DNA, 42 bp, Homo sapiens
  source 1..42: mol_type = other DNA
tgtgccagcagttacgacagtgggaccggggagctgtttttt

SEQ ID NO: 141 - DNA, 42 bp, Homo sapiens
  source 1..42: mol_type = other DNA
tgtgccagcagttacgactcagggaccggggagctgtttttt

SEQ ID NO: 142 - DNA, 36 bp, Homo sapiens
  source 1..36: mol_type = other DNA
tgtgcagagagctcgccgcaaggcaaactaatcttt

SEQ ID NO: 143 - DNA, 42 bp, Homo sapiens
  source 1..42: mol_type = other DNA
tgtgcagcaagacttaccggcactgccagtaaactcaccttt

SEQ ID NO: 144 - DNA, 42 bp, Homo sapiens
  source 1..42: mol_type = other DNA
tgcagcgttgggtccgggggcactaatgaaaaactgtttttt

SEQ ID NO: 145 - DNA, 324 bp, Homo sapiens
  source 1..324: mol_type = other DNA
atggagaccctcttgggcctgcttatcctttggctgcagctgcaatgggtgagcagcaaacaggaggtgacacagattcctgcagctctgagtgtcccagaaggagaaaacttggttctcaactgcagtttcactgatagcgctatttacaacctccagtggtttaggcaggaccctgggaaaggtctcacatctctgttgcttattcagtcaagtcagagagagcaaacaagtggaagacttaatgcctcgctggataaatcatcaggacgtagtactttatacattgcagcttctcagcctggtgactcagccacctacctc

SEQ ID NO: 146 - DNA, 39 bp, Homo sapiens
  source 1..39: mol_type = other DNA
tgtgctgtcttaatggatagcaactatcagttaatctgg

SEQ ID NO: 147 - DNA, 45 bp, Homo sapiens
  source 1..45: mol_type = other DNA
tgtgcctttatgcccagaggctcaaccctggggaggctatacttt

SEQ ID NO: 148 - DNA, 42 bp, Homo sapiens
  source 1..42: mol_type = other DNA
tgtgcagcaaggaatgccggcactgccagtaaactcaccttt

SEQ ID NO: 149 - DNA, 333 bp, Homo sapiens
  source 1..333: mol_type = other DNA
atgctgactgccagcctgttgagggcagtcatagcctccatctgtgttgtatccagcatggctcagaaggtaactcaagcgcagactgaaatttctgtggtggagaaggaggatgtgaccttggactgtgtgtatgaaacccgtgatactacttattacttattctggtacaagcaaccaccaagtggagaattggttttccttattcgtcggaactcttttgatgagcaaaatgaaataagtggtcggtattcttggaacttccagaaatccaccagttccttcaacttcaccatcacagcctcacaagtcgtggactcagcagtatacttc

SEQ ID NO: 150 - DNA, 330 bp, Homo sapiens
  source 1..330: mol_type = other DNA
atgaaaaagcatctgacgaccttcttggtgattttgtggctttatttttatagggggaatggcaaaaaccaagtggagcagagtcctcagtccctgatcatcctggagggaaagaactgcactcttcaatgcaattatacagtgagccccttcagcaacttaaggtggtataagcaagatactgggagaggtcctgtttccctgacaatcatgactttcagtgagaacacaaagtcgaacggaagatatacagcaactctggatgcagacacaaagcaaagctctctgcacatcacagcctcccagctcagcgattcagcctcctacatc

SEQ ID NO: 151 - DNA, 567 bp, Homo sapiens
  source 1..567: mol_type = other DNA
gggccgggcaccaggctcacggtcacagaggacctgaaaaacgtgttcccacccgaggtcgctgtgtttgagccatcagaagcagagatctcccacacccaaaaggccacactggtgtgcctggccacaggcttctaccccgaccacgtggagctgagctggtgggtgaatgggaaggaggtgcacagtggggtcagcacagacccgcagcccctcaaggagcagcccgccctcaatgactccagatactgcctgagcagccgcctgagggtctcggccaccttctggcagaacccccgcaaccacttccgctgtcaagtccagttctacgggctctcggagaatgacgagtggacccaggatagggccaaacctgtcacccagatcgtcagcgccgaggcctggggtagagcagactgtggcttcacctccgagtcttaccagcaaggggtcctgtctgccaccatcctctatgagatcttgctagggaaggccaccttgtatgccgtgctggtcagtgccctcgtgctgatggccatggtcaagagaaaggattccagaggctag

SEQ ID NO: 152 - DNA, 42 bp, Homo sapiens
  source 1..42: mol_type = other DNA
tgtgcagcaaggaataccggcactgccagtaaactcaccttt

SEQ ID NO: 153 - DNA, 456 bp, Homo sapiens
  source 1..456: mol_type = other DNA
gggaaggggaccaaactctcggtcataccaaatatccagaaccctgaccctgccgtgtaccagctgagagactctaaatccagtgacaagtctgtctgcctattcaccgattttgattctcaaacaaatgtgtcacaaagtaaggattctgatgtgtatatcacagacaaaactgtgctagacatgaggtctatggacttcaagagcaacagtgctgtggcctggagcaacaaatctgactttgcatgtgcaaacgccttcaacaacagcattattccagaagacaccttcttccccagcccagaaagttcctgtgatgtcaagctggtcgagaaaagctttgaaacagatacgaacctaaactttcaaaacctgtcagtgattgggttccgaatcctcctcctgaaagtggccgggtttaatctgctcatgacgctgcggctgtggtccagctga

SEQ ID NO: 154 - DNA, 327 bp, Homo sapiens
  source 1..327: mol_type = other DNA
atgagcatcggcctcctgtgctgtgcagccttgtctctcctgtgggcaggtccagtgaatgctggtgtcactcagaccccaaaattccaggtcctgaagacaggacagagcatgacactgcagtgtgcccaggatatgaaccatgaatacatgtcctggtatcgacaagacccaggcatggggctgaggctgattcattactcagttggtgctggtatcactgaccaaggagaagtccccaatggctacaatgtctccagatcaaccacagaggatttcccgctcaggctgctgtcggctgctccctcccagacatctgtgtacttc

SEQ ID NO: 155 - DNA, 36 bp, Homo sapiens
  source 1..36: mol_type = other DNA
tgtgcagagagtactccgggaggaaagcttatcttc

SEQ ID NO: 156 - DNA, 48 bp, Homo sapiens
  source 1..48: mol_type = other DNA
tgcgccagcagcttggagggtcaggccagctcctacgagcagtacttc

SEQ ID NO: 157 - DNA, 42 bp, Homo sapiens
  source 1..42: mol_type = other DNA
tgtgccagcagttttcttagcggcacagatacgcagtatttt

SEQ ID NO: 158 - DNA, 456 bp, Homo sapiens
  source 1..456: mol_type = other DNA
gggactggaacaagacttcaggtcacgctcgatatccagaaccctgaccctgccgtgtaccagctgagagactctaaatccagtgacaagtctgtctgcctattcaccgattttgattctcaaacaaatgtgtcacaaagtaaggattctgatgtgtatatcacagacaaaactgtgctagacatgaggtctatggacttcaagagcaacagtgctgtggcctggagcaacaaatctgactttgcatgtgcaaacgccttcaacaacagcattattccagaagacaccttcttccccagcccagaaagttcctgtgatgtcaagctggtcgagaaaagctttgaaacagatacgaacctaaactttcaaaacctgtcagtgattgggttccgaatcctcctcctgaaagtggccgggtttaatctgctcatgacgctgcggctgtggtccagctga